European Patent Application EP 4 317 459 A1, published February 7, 2024. Title: METHOD FOR THE DETECTION OF SARS-COV-2 BY DIGITAL PCR. Applicant: NATIONAL AND KAPODISTRIAN UNIVERSITY OF ATHENS. The sequence listing filed with the application follows.

SEQUENCE LISTING (20 sequences)

SEQ ID NO: 1 - DNA, 240 bp, SARS-COV-2
  source 1..240: mol_type = genomic DNA
gtttggtggaccctcagattcaactggcagtaaccagaatggagaacgcagtggggcgcgatcaaaacaacgtcggccccaaggtttacccaataatactgcgtcttggttcaccgctctcactcaacatggcaaggaagaccttaaattccctcgaggacaaggcgttccaattaacaccaatagcagtccagatgaccaaattggctactaccgaagagctaccagacgaattcgtgg

SEQ ID NO: 2 - DNA, 240 bp, SARS-COV-2
  source 1..240: mol_type = genomic DNA
ttcaactccaggcagcagtaggggaacttctcctgctagaatggctggcaatggcggtgatgctgctcttgctttgctgctgcttgacagattgaaccagcttgagagcaaaatgtctggtaaaggccaacaacaacaaggccaaactgtcactaagaaatctgctgctgaggcttctaagaagcctcggcaaaaacgtactgccactaaagcatacaatgtaacacaagctttcggcag

SEQ ID NO: 3 - DNA, 240 bp, SARS-COV-2
  source 1..240: mol_type = genomic DNA
aatgtcgcgcattggcatggaagtcacaccttcgggaacgtggttgacctacacaggtgccatcaaattggatgacaaagatccaaatttcaaagatcaagtcattttgctgaataagcatattgacgcatacaaaacattcccaccaacagagcctaaaaaggacaaaaagaagaaggctgatgaaactcaagccttaccgcagagacagaagaaacagcaaactgtgactcttcttcc

SEQ ID NO: 4 - RNA, 119 nt, synthetic construct
  source 1..119: mol_type = other RNA
ctttctgacatagaccagtagtgttgtccttcccgcccactaccatcctcatccacatatccctacaaataaggacaacgtagaggatggttgtcgccgattacagtccaaaaaaaaaa

SEQ ID NO: 5 - DNA, 19 bp, SARS-COV-2
  source 1..19: mol_type = other DNA
gcgatcaaaacaacgtcgg

SEQ ID NO: 6 - DNA, 23 bp, SARS-COV-2
  source 1..23: mol_type = other DNA
ggtcatctggactgctattggtg

SEQ ID NO: 7 - DNA, 29 bp, SARS-COV-2
  source 1..29: mol_type = other DNA
cccaaggtttacccaataatactgcgtct

SEQ ID NO: 8 - DNA, 20 bp, SARS-COV-2
  source 1..20: mol_type = other DNA
tgatgctgctcttgctttgc

SEQ ID NO: 9 - DNA, 24 bp, SARS-COV-2
  source 1..24: mol_type = other DNA
gatttcttagtgacagtttggcct

SEQ ID NO: 10 - DNA, 28 bp, SARS-COV-2
  source 1..28: mol_type = other DNA
ctgcttgacagattgaaccagcttgaga

SEQ ID NO: 11 - DNA, 24 bp, SARS-COV-2
  source 1..24: mol_type = other DNA
ttggatgacaaagatccaaatttc

SEQ ID NO: 12 - DNA, 22 bp, SARS-COV-2
  source 1..22: mol_type = other DNA
ggcttgagtttcatcagccttc

SEQ ID NO: 13 - DNA, 29 bp, SARS-COV-2
  source 1..29: mol_type = other DNA
caaaacattcccaccaacagagcctaaaa

SEQ ID NO: 14 - DNA, 25 bp, SARS-COV-2
  source 1..25: mol_type = other DNA
catagaccagtagtgttgtccttcc

SEQ ID NO: 15 - DNA, 20 bp, SARS-COV-2
  source 1..20: mol_type = other DNA
actgtaatcggcgacaacca

SEQ ID NO: 16 - DNA, 28 bp, SARS-COV-2
  source 1..28: mol_type = other DNA
ccactaccatcctcatccacatatccct

SEQ ID NO: 17 - DNA, 20 bp, SARS-COV-2
  source 1..20: mol_type = other DNA
gcctgccgtgtgaaccatgt

SEQ ID NO: 18 - DNA, 22 bp, SARS-COV-2
  source 1..22: mol_type = other DNA
aaatgcggcatcttcaaacctc

SEQ ID NO: 19 - DNA, 30 bp, SARS-COV-2
  source 1..30: mol_type = other DNA
catgatgctgcttacatgtctcgatcccac

SEQ ID NO: 20 - RNA, 130 nt, Homo sapiens
  source 1..130: mol_type = mRNA
aaaaagatgagtatgcctgccgtgtgaaccatgtgactttgtcacagcccaagatagttaagtgggatcgagacatgtaagcagcatcatggaggtttgaagatgccgcatttggattggatgaattcca